European Patent Application EP 4 286 397 A1, published December 6, 2023. Title: HYDROGEL-FORMING PROTEINS. Applicant: ETH Zürich. The sequence listing filed with the application follows.

SEQUENCE LISTING (77 sequences)

SEQ ID NO: 1 - protein, 8 aa, Artificial Sequence
  Artificial sequence
AEAEAKAK

SEQ ID NO: 2 - protein, 8 aa, Artificial Sequence
  Artificial sequence
AEAKAEAK

SEQ ID NO: 3 - protein, 8 aa, Artificial Sequence
  Artificial sequence
RADARADA

SEQ ID NO: 4 - protein, 8 aa, Artificial Sequence
  Artificial sequence
RARADADA

SEQ ID NO: 5 - protein, 8 aa, Artificial Sequence
  Artificial sequence
RAEARAEA

SEQ ID NO: 6 - protein, 16 aa, Artificial Sequence
  Artificial sequence
RAEARAEARAEARAEA

SEQ ID NO: 7 - protein, 8 aa, Artificial Sequence
  Artificial sequence
KADAKADA

SEQ ID NO: 8 - protein, 8 aa, Artificial Sequence
  Artificial sequence
KAKADADA

SEQ ID NO: 9 - protein, 8 aa, Artificial Sequence
  Artificial sequence
AEAEAHAH

SEQ ID NO: 10 - protein, 8 aa, Artificial Sequence
  Artificial sequence
FEFKFEFK

SEQ ID NO: 11 - protein, 8 aa, Artificial Sequence
  Artificial sequence
FEFEFKFK

SEQ ID NO: 12 - protein, 8 aa, Artificial Sequence
  Artificial sequence
LELKLELK

SEQ ID NO: 13 - protein, 8 aa, Artificial Sequence
  Artificial sequence
LELELKLK

SEQ ID NO: 14 - protein, 8 aa, Artificial Sequence
  Artificial sequence
HEHEHKHK

SEQ ID NO: 15 - protein, 8 aa, Artificial Sequence
  Artificial sequence
VEVKVEVK

SEQ ID NO: 16 - protein, 16 aa, Artificial Sequence
  Artificial sequence
KAKAKAKAEAEAEAEA

SEQ ID NO: 17 - protein, 16 aa, Artificial Sequence
  Artificial sequence
EAEAEAEAKAKAKAKA

SEQ ID NO: 18 - protein, 16 aa, Artificial Sequence
  Artificial sequence
RARARARADADADADA

SEQ ID NO: 19 - protein, 16 aa, Artificial Sequence
  Artificial sequence
ADADADADARARARAR

SEQ ID NO: 20 - protein, 16 aa, Artificial Sequence
  Artificial sequence
DADADADARARARARA

SEQ ID NO: 21 - protein, 7 aa, Artificial Sequence
  Artificial sequence
GSGSGSG

SEQ ID NO: 22 - protein, 9 aa, Artificial Sequence
  Artificial sequence
GSGSGSGSG

SEQ ID NO: 23 - protein, 11 aa, Artificial Sequence
  Artificial sequence
GSGSGSGRGDS

SEQ ID NO: 24 - protein, 12 aa, Artificial Sequence
  Artificial sequence
GSGSGSGPHSRN

SEQ ID NO: 25 - protein, 13 aa, Artificial Sequence
  Artificial sequence
GSGSGSGPHSRNS

SEQ ID NO: 26 - protein, 13 aa, Artificial Sequence
  Artificial sequence
GSGSGSGSGRGDS

SEQ ID NO: 27 - protein, 11 aa, Artificial Sequence
  Artificial sequence
GKGSGSGRGDS

SEQ ID NO: 28 - protein, 4 aa, Artificial Sequence
  Artificial sequence
  MISC_FEATURE (4)..(4): X is any amino acid
RGDX

SEQ ID NO: 29 - protein, 4 aa, Artificial Sequence
  Artificial sequence
RGDS

SEQ ID NO: 30 - protein, 6 aa, Artificial Sequence
  Artificial sequence
GRGDSP

SEQ ID NO: 31 - protein, 5 aa, Artificial Sequence
  Artificial sequence
PHSRN

SEQ ID NO: 32 - protein, 6 aa, Artificial Sequence
  Artificial sequence
PHSRNS

SEQ ID NO: 33 - protein, 4 aa, Artificial Sequence
  Artificial sequence
REDV

SEQ ID NO: 34 - protein, 5 aa, Artificial Sequence
  Artificial sequence
IKVAV

SEQ ID NO: 35 - protein, 5 aa, Artificial Sequence
  Artificial sequence
YIGSR

SEQ ID NO: 36 - protein, 7 aa, Artificial Sequence
  Artificial sequence
RYVVLPR

SEQ ID NO: 37 - protein, 10 aa, Artificial Sequence
  Artificial sequence
RNIAEIIKDI

SEQ ID NO: 38 - protein, 16 aa, Artificial Sequence
  Artificial sequence
CKAAKRPKAAKDKQTK

SEQ ID NO: 39 - protein, 10 aa, Artificial Sequence
  Artificial sequence
SGESPAYYTA

SEQ ID NO: 40 - protein, 8 aa, Artificial Sequence
  Artificial sequence
GPQGIAGQ

SEQ ID NO: 41 - protein, 8 aa, Artificial Sequence
  Artificial sequence
CPQGIWGQ

SEQ ID NO: 42 - protein, 8 aa, Artificial Sequence
  Artificial sequence
GDQGIAGF

SEQ ID NO: 43 - protein, 8 aa, Artificial Sequence
  Artificial sequence
VPMSMRGG

SEQ ID NO: 44 - protein, 7 aa, Artificial Sequence
  Artificial sequence
VMPSMRG

SEQ ID NO: 45 - protein, 6 aa, Artificial Sequence
  Artificial sequence
VPMSMR

SEQ ID NO: 46 - protein, 6 aa, Artificial Sequence
  Artificial sequence
RPMSMR

SEQ ID NO: 47 - protein, 8 aa, Artificial Sequence
  Artificial sequence
IPVSLRSG

SEQ ID NO: 48 - protein, 8 aa, Artificial Sequence
  Artificial sequence
RPFSMIMG

SEQ ID NO: 49 - protein, 8 aa, Artificial Sequence
  Artificial sequence
VPLSLYSG

SEQ ID NO: 50 - protein, 8 aa, Artificial Sequence
  Artificial sequence
IPESLRAG

SEQ ID NO: 51 - protein, 6 aa, Artificial Sequence
  Artificial sequence
PAYYTA

SEQ ID NO: 52 - protein, 8 aa, Artificial Sequence
  Artificial sequence
YAAPVRGG

SEQ ID NO: 53 - protein, 8 aa, Artificial Sequence
  Artificial sequence
GTAGLIGQ

SEQ ID NO: 54 - protein, 8 aa, Artificial Sequence
  Artificial sequence
GMGPSGPN

SEQ ID NO: 55 - protein, 7 aa, Artificial Sequence
  Artificial sequence
GTARSAS

SEQ ID NO: 56 - protein, 7 aa, Artificial Sequence
  Artificial sequence
TSHRSAS

SEQ ID NO: 57 - protein, 7 aa, Artificial Sequence
  Artificial sequence
DRIRSAS

SEQ ID NO: 58 - protein, 254 aa, Artificial Sequence
  Artificial sequence
HHHHHHGSGSAEAEAKAKAEAEAKAKAEAEAKAKAEAEAKAKAEAEAKAKAEFGSGSGSGRGDSGSGSGSGRGDSGSGSGSGRGDSGSGSGSGRGDSGSGSGSGRGDSWAEAEAKAKAEAEAKAKAEAEAKAKAEAEAKAKAEAEAKAKDWGSGSGSGRGDSGSGSGSGRGDSGSGSGSGRGDSGSGSGSGRGDSGSGSGSGRGDSPRGAEAEAKAKAEAEAKAKAEAEAKAKAEAEAKAKAEAEAKAKGTSGS

SEQ ID NO: 59 - protein, 223 aa, Artificial Sequence
  Artificial sequence
HHHHHHGSGSAEAEAKAKAEAEAKAKAEAEAKAKAEAEAKAKAEAEAKAKAEFGSGSGSGPHSRNSGSGSGSGSGRGDSGSGSGSGPHSRNSGSGSGSGSGRGDSGSGWAEAEAKAKAEAEAKAKAEAEAKAKDWGSGSGSGRGDSGSGSGSGPHSRNSGSGSGSGSGRGDSGSGPRGAEAEAKAKAEAEAKAKAEAEAKAKAEAEAKAKAEAEAKAKGTSGS

SEQ ID NO: 60 - protein, 254 aa, Artificial Sequence
  Artificial sequence
HHHHHHGSGSAEAEAKAKAEAEAKAKAEAEAKAKAEAEAKAKAEAEAKAKAEFGSGSGSGPHSRNSGSGSGSGSGRGDSGSGSGSGPHSRNSGSGSGSGSGRGDSGSGWAEAEAKAKAEAEAKAKAEAEAKAKAEAEAKAKAEAEAKAKDWGSGSGSGPHSRNSGSGSGSGSGRGDSGSGSGSGPHSRNSGSGSGSGSGRGDSGSGPRGAEAEAKAKAEAEAKAKAEAEAKAKAEAEAKAKAEAEAKAKGTSGS

SEQ ID NO: 61 - protein, 244 aa, Artificial Sequence
  Artificial sequence
AEAEAKAKAEAEAKAKAEAEAKAKAEAEAKAKAEAEAKAKAEFGSGSGSGPHSRNSGSGSGSGSGRGDSGSGSGSGPHSRNSGSGSGSGSGRGDSGSGWAEAEAKAKAEAEAKAKAEAEAKAKAEAEAKAKAEAEAKAKDWGSGSGSGPHSRNSGSGSGSGSGRGDSGSGSGSGPHSRNSGSGSGSGSGRGDSGSGPRGAEAEAKAKAEAEAKAKAEAEAKAKAEAEAKAKAEAEAKAKGTSGS

SEQ ID NO: 62 - protein, 213 aa, Artificial Sequence
  Artificial sequence
AEAEAKAKAEAEAKAKAEAEAKAKAEAEAKAKAEAEAKAKAEFGSGSGSGPHSRNSGSGSGSGSGRGDSGSGSGSGPHSRNSGSGSGSGSGRGDSGSGWAEAEAKAKAEAEAKAKAEAEAKAKDWGSGSGSGRGDSGSGSGSGPHSRNSGSGSGSGSGRGDSGSGPRGAEAEAKAKAEAEAKAKAEAEAKAKAEAEAKAKAEAEAKAKGTSGS

SEQ ID NO: 63 - protein, 250 aa, Artificial Sequence
  Artificial sequence
MRGSHHHHHHGSGSAEAEAKAKAEAEAKAKAEAEAKAKAEAEAKAKAEAEAKAKAEFGSGSGSGRGDSGSGESPAYYTAGSGSGSGRGDSGSGSGSGRGDSGSGSGSGRGDSWAEAEAKAKAEAEAKAKAEAEAKAKAEAEAKAKAEAEAKAKDWGSGSGSGRGDSGSGSGSGRGDSGSGSGSGRGDSGSGSGSGRGDSGSGSGSGRGDSPRGAEAEAKAKAEAEAKAKAEAEAKAKAEAEAKAKGTSGS

SEQ ID NO: 64 - protein, 258 aa, Artificial Sequence
  Artificial sequence
MRGSHHHHHHGSGSAEAEAKAKAEAEAKAKAEAEAKAKAEAEAKAKAEAEAKAKAEFGKGSGSGRGDSGSGSGSGRGDSGSGSGSGRGDSGSGSGSGRGDSGSGSGSGRGDSWAEAEAKAKAEAEAKAKAEAEAKAKAEAEAKAKAEAEAKAKDWGSGSGSGRGDSGSGSGSGRGDSGSGSGSGRGDSGSGSGSGRGDSGSGSGSGRGDSPRGAEAEAKAKAEAEAKAKAEAEAKAKAEAEAKAKAEAEAKAKGTSGS

SEQ ID NO: 65 - protein, 258 aa, Artificial Sequence
  Artificial sequence
MRGSHHHHHHGSGSAEAEAKAKAEAEAKAKAEAEAKAKAEAEAKAKAEAEAKAKAEFGKGSGSGRGDSGSGSGSGRGDSGSGSGSGRGDSGSGSGSGRGDSGSGSGSGRGDSWAEAEAKAKAEAEAKAKAEAEAKAKAEAEAKAKAEAEAKAKDWGKGSGSGRGDSGSGSGSGRGDSGSGSGSGRGDSGSGSGSGRGDSGSGSGSGRGDSPRGAEAEAKAKAEAEAKAKAEAEAKAKAEAEAKAKAEAEAKAKGTSGS

SEQ ID NO: 66 - protein, 178 aa, Artificial Sequence
  Artificial sequence
HHHHHHGSGSAEAEAKAKAEAEAKAKAEAEAKAKAEAEAKAKAEAEAKAKAEFGSGSGSGRGDSGSGSGSGRGDSGSGSGSGRGDSGSGSGSGRGDSGSGSGSGRGDSGSGSGSGRGDSGSGSGSGRGDSPRGAEAEAKAKAEAEAKAKAEAEAKAKAEAEAKAKAEAEAKAKGTSGS

SEQ ID NO: 67 - protein, 179 aa, Artificial Sequence
  Artificial sequence
HHHHHHGSGSAEAEAKAKAEAEAKAKAEAEAKAKAEAEAKAKAEAEAKAKAEFWGSGSGSGRGDSGSGSGSGRGDSGSGSGSGRGDSGSGSGSGRGDSGSGSGSGRGDSGSGSGSGRGDSGSGSGSGRGDSPRGAEAEAKAKAEAEAKAKAEAEAKAKAEAEAKAKAEAEAKAKGTSGS

SEQ ID NO: 68 - protein, 168 aa, Artificial Sequence
  Artificial sequence
AEAEAKAKAEAEAKAKAEAEAKAKAEAEAKAKAEAEAKAKAEFGSGSGSGRGDSGSGSGSGRGDSGSGSGSGRGDSGSGSGSGRGDSGSGSGSGRGDSGSGSGSGRGDSGSGSGSGRGDSPRGAEAEAKAKAEAEAKAKAEAEAKAKAEAEAKAKAEAEAKAKGTSGS

SEQ ID NO: 69 - protein, 5 aa, Artificial Sequence
  Artificial sequence
GTSGS

SEQ ID NO: 70 - protein, 7 aa, Artificial Sequence
  Artificial sequence
  MISC_FEATURE (2)..(2): X is any amino acid, unless otherwise defined
GXGSGSG

SEQ ID NO: 71 - protein, 11 aa, Artificial Sequence
  Artificial sequence
  MISC_FEATURE (2)..(2): X is any amino acid, unless otherwise defined
GXGSGSGRGDS

SEQ ID NO: 72 - protein, 7 aa, Artificial Sequence
  Artificial sequence
GKGSGSG

SEQ ID NO: 73 - protein, 4 aa, Artificial Sequence
  Artificial sequence
GSGW

SEQ ID NO: 74 - protein, 6 aa, Artificial Sequence
  Artificial sequence
GSGPRG

SEQ ID NO: 75 - protein, 4 aa, Artificial Sequence
  Artificial sequence
AEFW

SEQ ID NO: 76 - protein, 4 aa, Artificial Sequence
  Artificial sequence
GSGS

SEQ ID NO: 77 - protein, 10 aa, Artificial Sequence
  Artificial sequence
HHHHHHGSGS